European Patent Application EP 4 306 104 A1, published January 17, 2024. Title: Pharmaceutical Composition for Preventing or Treating Viral Infection Comprising Polymer Nanodiscs. Applicant: MVRIX Co.,Ltd. The sequence listing filed with the application follows.

SEQUENCE LISTING (4 sequences)

SEQ ID NO: 1 - DNA, 33 bp, Artificial Sequence
  plasmid forward primer
tgtggctcctgttgttaaaagtttgatgaggat

SEQ ID NO: 2 - DNA, 33 bp, Artificial Sequence
  plasmid reverse primer
atcctcatcaaacttttaacaacaggagccaca

SEQ ID NO: 3 - DNA, 26 bp, Artificial Sequence
  mCherry-Luciferase viral RNA forward primer
gggggtgggaagccctcaaatattgg

SEQ ID NO: 4 - DNA, 23 bp, Artificial Sequence
  mCherry-Luciferase viral RNA reverse primer
gggttgtgccgcctttgcaggtg